European Patent Specification EP 3 022 297 B1, published July 5, 2023. Title: Genetically stable oncolytic RNA virus, method of manufacturing and use thereof. Applicant: SIA Latima. Application EP13176757. The sequence listing filed with the application follows.

SEQUENCE LISTING (55 sequences)

SEQ ID NO: 1 - RNA, 7427 nt, Enterovirus sp. Echo 7
  CDS (743)-(7327): Modified virus
uuaaaacagccuguggguuguucccacccacagggcccacugggcgcuagcacacugguaucacgguacccuugugcgccuguuuuaucuuccccuccccacuguaacuuagaagaaugacauaaacggucaacagauagcucaguacaccaacugagccccgaccaagcacuucuguuaccccggaccgaguaacaauaggcugcucgcgcggcugaaggugaaaacguucguuacccggccaauuacuucgagaaaccuaguaccaccaugaagguugcgcagcguuucgcuccgcacaaccccaguguagaucaggucgaugagucaccgcacuccccacgggcgaccguggcgguggcugcgcuggcggccugccuauggggcaacccaugggacgcuucaauacugacauggugcgaagagucuauugagcuaauugguaguccuccggccccugaaugcggcuaauccuaacugcggggcaagugcccacaaaccaguggguggcuugucguaacggguaacccugcagcggaaccgacuacuuuggguguccguguuuccuuuuauucuuauucuggcugcuuauggugacaauugagagauuguurccauauagcuauuggauuggccrucuggugaguaacagagcaaucauauuccucuuuguuggauuuauaccacuugauuccacuaguuacaacacucugcuacauauuauuugcuuaaauacaagaagaugggagcacaaguaucgacacaaaagacuggugcacacgagaccsguuugagcgcuaacggacacucuaucauucacuauaccaacaucaacuacuacaaagaugcagcauccaacucagccaacaggcaggauuucacccaggauccagguaaguucacugaaccggucaaggauaucaugaucaaaucgaugcccgcccuaaacucaccguccgcggaggagugcggguacagcgacagggugagaucccuaacgcucggcaacucaaccauuaccacucaagaaagugcaaacguaguuguuggcuauggcagguggccagaguacuugaaagaugaagaagcuacugcggaagaucagccaacacaacccgauguagccacrugcagguucuacacguuggaauccguccagugggagaaaaauagcgcuggauggugguggaaguuccccgaagcacuuaaggacaugggccucuuuggucagaacaugcuuuaccacuaucucgguagagcaggcuacacuauacaugugcagugcaacgcauccaaauuucaucagggcugucuacuuguugucuguguaccugaagcugagaugggguguucccagacggacaaagagguugcugcgaugaaccucacgaagggugaaacggcgcacaaguuugaaccaaccaaaaccacaggcggccacacagugcaauccauagugugcaacgcggguaugggcaucggcguggggaaccucaccaucuacccucaccaguggaucaacuugcgcacuaauaacugcgcuacaauugugaugccguauauaaauucaguacccauggauaacauguuuaggcacuacaauuucacgcuaauggugaucccauuugcaccccuggauuacaaugcccaagcaucugaguacguaccuguaacugucacaauagccccaaugugugcagaauacaaugguuuaaggcuggcuuaccagcaagggcugccagugcuaaauacaccgggaagcaaucaguuuaugacaucggaugauuuucaauccccuucggcuaugccacaauuugaugugacuccgcacauggacaucccaggugaagugcacaaccucauggagauugcagaaguugauucggugguaccuguuaacaacacugcggccaaucugcaaagcauggacgcauaucacauagaggugaacrcaggaaaucaccaaggugaaaagauauucgcuuuccagauacaacccgggcuggauucaguguuuaagagaacacugcuaggugaagugcucaauuauuacgcgcacuggucagggagcauuaagcuaacauucacauuuugugguucagcaauggccacgggcaagcuacucuuagcauacuccccaccuggcgccgauguaccggcuagcagaaagcaggcaaugaugggaacccauaucaucugggacuuagggcugcaauccaguugcguucuauguauuccauggaucagucagacacauuaucgccuagugcaacaggaugaguacaccagcgccggcaaugucaccugcugguaucagacagguauagugguuccacccggcacacccaacaagugugucguccugugcuuugugucagcguguaaugacuucuccgugcgcaugcugcgugacacaccauucaucggccaaacaacacugcuacaaggugauacggacguggccgucaacaaugcaguagccaggguagcugauacaauugccagugggcccagcaacuccacuagcauuccugcacuaaccgcaguugagacugggcacacaucacagguagagccuagugauacaaugcaaacacggcauguaaagaacuaccauucgcgaucugaaucaacaauagagaacuuccuuagccggucggccuguguauauauugaagaguacuuuaccaaagaucaagacagcgccaauagguacaugucauggacuauaaaugcuagaaggauggugcaauugaggcgaaaguuugaacuguucacauacaugcgguuugauauggagaucacauuuguuaucacuaguagacaacugccugggacuagcaucgcgcaagacaugccgccacugacacaccaaaucauguauauacccccuggugguccaguaccaaacagugugaccgauuuugcauggcaaacuucgacuaauccaaguaucuuuuggacugagggcaaugcccccccgcguauguccauaccauuuauaagcauagggaaugcauacagcaacuuuuaugacggruggucgcacuucucacaaaaugggguauacggcuacaaugcauuaaacaacaugggcaaauuauacgcacgccaugugaacaaagacacaccguaccagauguccaguacgauucguguguacuuuaaacccaaacauaucagagugugggugccaagaccaccacguuugugccccuauauuaaaucuaguaacguuaacuuugacccaaccaaccuaacugauucaagaucaaguauaacauaugugccagacacuauccguccggaaguccguacagcuggaaaauucggccaccaguccggugcuguuuacguggguaauuacagaauagugaacaggcaccucgccacgcacaacgacuggcaaaacugugugugggaagacuacaacagagaccuccuugugagcaccacuacagcccaugggugugacacuauagccagaugucagugcacagcaggcguauauuuuugugccucaaggaacaaacauuacccagucaccuucgaggggccaggcuugguggaaguucaggagagcgaguacuacccaaaaagayaucagucccacgugcuucuagcugcaggauuuucugaaccgggcgauuguggcggaauccucagaugucaacacggcgugaucgguaucgucaccauggguggagagggggucguuggguuugccgacgucagagaccuacugugguuagaggaugaugccauggaacagggcguaagagacuauguugaacaacuaggaaaugcuuucggcucagguuucaccaaucaaauuugugaacaggucaaccuccucaaagagucauugguuggacaggauucuauucuggaaaaaucccuuaaggcucuaguuaagauuaucucagcacuggucruuguagugagaaaucacgaugaucucauaacgguuaccgccacucuagcuuuaauugguugcaccucuucuccguggcgguggcucaagcagaaggugucacaauauuauggaauacccagggccgagcgacaaaacaauagcuggcucaagaaguuuacugagaugaccaacgccugcaagggcauggaguggauagccauaaaaauucaaaaguuuauugaguggcuuaaagucaagauucugccggaagugaaggaaaaacacgaguuccucaacaggcuaaagcaauuaccacuccuagagagccagauugcaaccauagagcagagugcaccaucgcagagugaucaagagcaacucuucuccaacguccaguacuucgcccauuauugcagaaaguaugcgccauuguacgcugccgaagcgaagagaguguucucacuugagaagaaaaugagcaacuacauacaguucaaguccaaaugccguauugagccuguaugcuuacuccuacauggcagcccaggggccggaaaguccguggccaccaacuugauuggcagaucccucgcagaaaaacucaacagcucuguruacucccuaccaccagaccccgaccacuuugacggcuacaagcagcaagcggucgugaucauggaugacuuaugccaaaauccugauggaaaagaugucucacuauuuugucagaugguuucuagcguggacuuuguaccaccgauggcugcgcuagaggaaaaaggaauccuauuuaccuccccguucguguuggcaucaaccaacgcuggguccaucaaugcacccacugugucugacagcagagcgcucgcuaggagauuccacuuugacaugaacauugaagucauuucuauguacagucaaaacggcaagaucaacaugcccaugucaguuaaaacaugugaugaagaguguuguccaguuaacuucaaaaggugcugcccguugguguguggaaaggcyaugcaauucauugauaggagaacucaaguuagauauucgcuggacaugcuaguuacugaaauguuuagggaguauaaccauagacacagugugggagccacucuugaagcucuguuccaagggccaccagucuacagagagaucaaaaucagcgucgccccagagacacccccaccaccagcuauugcugauuuacugaaaucaguggacagugaagcugugagggaauacugcaaggagagaggguggcuugugccagagaucaauucuacccuacaaauagagaagcaugugaguagagcauucauauguuuacaagcccuaaccacguuuguuucaguugcugguauaauauacauuauuuacaaauuauuugcagguuuccaaggcgccuacacagggaugcccaaccagaaaccuaaggugcccacccugagacaggccaaaguacagggcccagcguuugaguucgcuguggcgaugaugaaaaggaacgccaguacaguaaaaaccgaguacggugaauucaccaugcuuggcauuuacgacaagugggcgguguuaccgcgccacgccaagccuggccccaccaucuugaugaaugaucaggaagucggcguguuggaugccaaggaacuaguugauaaagaugggacaaaucuagaauugacucuccugaagcucaaccguaacgaaaaguucagagauauuaggggguuucuagcaagagaagagguugaagugaaugaagcuguccuagcaauaaauacaagcaaauucccuaacauguacauaccagugggccaggugacugacuacggguuucugaaccugggagggacucccacgaagagaaugcucauguauaacuucccaacuagagcaggucaguguggagguguccucaugucaacagggaaaguccugggaauacauguaggagggaauggacaucaaggguucucagcggcacuccucaggcacuacuucaacgaggagcagggugaaauagaauucauugagagcucaaaggacgcgggauucccugugaucaacacucccaguaagacaaaauuggaaccaaguguguuucaccagguguucgagggcaacaaggaaccagcgguccuuagaaauggggacccacgacucaaagccaacuucgaggaagcaaucuucuccaaguacauuggcaaugucaacacgcauguagaugaguacauguuggaggcuguggaccauuaugcaggacaacuagcuacucuggacaucaguacggagcccaugaagcuagaggacgccguguaugguacagaggggcuggaagcacuagaccuaaccaccagugcaggcuacccuuacguggcccugggcaucaagaaaagagauauucuaucuaagaagacuaaagaccucacuaaguugaaggaaugcauggacaaauauggccuaaauuugccaaugguaaccuacgucaaagaugaguugagaucugcugagaagguggccaagggaaaauccaggcuuauugaggcuucuagucucaaugacucaguagcaaugaggcaaacauuuggaaauuuauauaagaccuuucaccucaacccgggcaucguuacgggcagugcuguugggugugauccagauguguuuuggagcaagaucccuguuaugcuugauggacaucucauagcuuuugacuauucaggcuaugacgcuagccucagcccagugugguuugcauguuugaaacuucuccuagagaaacuaggguauacaaacaaggaaacaaacuacauagauuaccucuguaauucccaucaccuguauagagacaagcacuacuuuguaagaggcgguaugccaucaggguguucaggcaccagcauauuuaauuccaugauuaacaacaucauaaucaggacucucaugcugaagguuuauaaaggcauugauuuggaccaauucagaaugauugccuauggggaugaugugauugcuuccuauccguggccuaucgaugcuucgcuguuagcugaagcaggaaaagauuaugguuuaaucaugaccccagcagacaaaggcgagugcuucaacgagguaaccuggacgaaugugaccuuucugaaaagguacuuuagggcagaugagcaauacccauuucugguccauccuguuaugccaaugaaggacauccaugagucuauuagguggaccaaagaucccaagaacacacaggaucaugugcgcucgcugugccuauuggcuuggcacaacggggagcaagaauaugaggaguuuauucgcaagaucagaagcgugcccguugggcgcugcuugacccuacccgcuuuuucaacacugcgcaggaaguggcuggacuccuuuuaaaauuagagcauaauuaguaaaucauaauuggcuuaacccuaccgcaugaaccgaacuugauaaaagugcgguagggguaaauucuccgcauucggugcgg

SEQ ID NO: 2 - RNA, 7434 nt, Enterovirus sp. Echo 7
  CDS (743)-(7333)
  unsure 4448: Unmodified (native) virus
uuaaaacagccuguggguuguucccacccacagggcccacugggcgcuagcacacugguaucacgguaccuuugugcgccuguuuuauaucccccuccccacuguaacuuagagaaaucacauaaacgaucaauagaaggcgcagcacaccagcugagucuugaccaagcacuucuguuuccccggacugaguaucaauagacugcucacgcgguugaaggagaaaacguucguuacccggccaacuacuucgagaaaccuaguaccaccaugaaaguugcgcaguguuucgcucagcacaaccccaguguagaucaggucgaugagucaccgcauuccccacgggcgaccguggcgguggcugcguuggcggccugccuauggggcaacccaugggacgcuucaauacugacauggugcgaagagucuauugagcuaguugguaguccuccggccccugaaugcggcuaauccuaacugcggagcaagugcccacaaaccaguggguagcuugucguaacgggcaacucugcagcggaaccgacuacuuuggguguccguguuuccuuuuauucuuauucuggcugcuuauggugacaauugagagauuguuaccauauagcuauuggauuggccauccggugacuaacagagcaaucauauuccucuuuguuggauuuauaccacuugauuccacuaguuacaacacucugcuacacauuauuuacuuaaaaccaagaagaugggagcacaaguaucaacacaaaaaacuggugcacaugagaccsguuugagcgcuaacggaagcuccaucauucacuacaccaacaucaauuacuacaaagaugcagcauccaacucagccaacaggcaagacuucacccaagauccaggcaaauucaccgaaccggucaaggauaucaugaucaagucgaugcccgcccuaaacucaccgaccguggaggaguguggguacagugauagggugagauccauaacgcucggcaacucaaccauuaccacucaggagagugcaaauguaguuguuggcuauggcggguggccagaguacuugaaagaugaagaagcuacugcggaagaucaaccaacacaacccgauguagccacaugcagguuuuacacgcuggaauccguccagugggagaaaaauuccgcuggauggugguggaaguuccccgaagcacuuaaggacaugggccucuuuggucaaaacaugcauuaccacuaccucgguagagcaggcuacacuauacacgugcagugcaaugcauccaaauuccaccaaggcugucuacuuguugucuguguaccugaggcugagaugggguguuccaaaguggacgguacuguaaaugagcaggaauugacggagggugaaacggauaugaagcuugaacccaccagaaccacaggcguacgccgagugcaauccgcaguguacaacgcggguaugggcgucggcguggggaaccucaccaucuucccucaccaguggaucaaccugcgcacuaacaacugugcuacaauugugaugccauacauaaauaguguacccauggauaacauguuuaggcacuacaacuucacgcuaaugaugaucccauuugcaccccuggauuacaccaaccaagcaucuacguacguaccuauaacugucacaauagcaccaaugugugcugaauacaaugguuugaggcucguuaccucgcaaggguugccagugaugaacacaccgggaagcaaucaguuccugacaucggaugacuuucaaucaccuucggcuaugccacaauuugaugugacuccagacauggacaucccaggugaagugaacaaccucauggagauugcagagguugacucggugguaccuguuaacaacaaugaggccaaucugaaaagcauggacgcauaccgcauaccggugaacrcaggaaaucaacaaggugaaaagauauuugguuuccaaauacaacccgggcuugauucaguguuuaagagaacacugcuaggugagaugcucaauuauuacacgcacuggucagggagcauuaagcuaacauuuauguuuugugguucagcaauggccacgggcaaauuacucuuagcauacucaccaccuggcgccgauguaccgacuagcagaaaggaggcaaugcugggaacccaugucaucugggacuuugggcugcaauccaguuguguucuguguguuccauggaucagccagacacacuacagguuggugcagcaggaugaguacaccggcgccggcuauaucaccugcugguaccaaacaaguauagugguuccacccggcacacccaaaaagugugucauccugugcuuugugucagcguguaaugauuucuccgugagcaugcugagugacacaccauucaucggccaaacagcacugcugcagagcccuguggaagaagcugaagagaacgcaguugcacguguggcugacacaauugccagugggcccagcaacuccgagagcguuccugcacuaacagcaguugagacugggcacacaucacagguagugccuagugacacaaugcaaacaaggcaugugaagaacuaccauucgagaucugagucaacaauagagaacuuccuuagcagguccgccuguguguauauugaagaguacuauaccaacacugaaaccagacaaaauuuauacauguugcccacuauaaauacuagauggauggugcaauugaggagaaaguuugagauguucacauacaugagguuugacauggaaaucacauuuguuaucacuaguagacaacugcaucgaacuagcaugccgcaggacaugccgguacugacacaccaaaucauguauguaccaccuggugguccaguaccaaacaguguggacgauuacgcauggcaaacuucgacuaacccaagugucuuuuggacugagggcaaugccccaccgcguauguccauaccauucauaagcauagggaaugcauacagcaacuuuuaugauggguccucgcacuucuuacaauaugggguauauggcuacaacacauuaaacaacauggggaaauuauacguacgccaugugaacaaccacacaccauaccaaaugaccaguacgguuaguguguacuuuaaacccaaacaugucagagcgugggugccgagaccaccacgucugugccccuacaaaaaugcauggaacguuaacuuugaaccaacaaacguaacugauucaagaucaaguaucacauauauuccugagacggucaaaccagaccuaucaaaagcuggagcuuucggccaccaguccggugcuguuuauguggguaacuacagaguggugaauaggcaccucgccacgcacaacgacuggcaaaacugugugugggaagacuacaacagagaccuccuugugagcaccaccacagcccaugggugugacaccauagccagaugccagugcacaacaggcguguacuuuugugccucaaggaacaaacacuacccagucaccuuugaggggccaggccugguggaaguucaggagagugaguacuacccaaaaagauaccaaucccaugugcuucuagcugcaggauuuucugaaccaggcgauugugguggaauccucaggugugaacauggugucaucgguaucgucaccauggguggagagggggucguuggguuugccgacguccgagaccuacugugguuagaggaugaugccauggaacagggcguaagagacuauguugaacaacuaggaaaugcuuuuggcucagguuucaccaaccaaauuugugaacaagucaaccuccucaaagagucacugguuggacaggacuccauucuggagaaaucccuuaaagcccuaguuaagauuaucucagcacuggucauuguagugagaaaucacgaugaccucaucacagugacugccacucuagcccucauugguugcaccucuucuccauggcgguggcucaaacagaaagugucacaauauuauggaauacccauggcugagcgacaaaacaauggcuggcucaagaaguucacugagaugaccaaugccugcaagggcauggaguggauagccaucaaaauucaaaaauuuauugaguggcuuaaagucaagaucuaccagaaguguaggaaaaacaugaguuccucaacagacuauaacaacuaccacucuuggaagagucagauugccaccauagaacaaagugcaccaucgcagagugaccaggagcaacuguuuuccaauguccaguacuucgcccacuauugcagaaaguaugcgccacuguaugcagcugaggcaaagagaguguucucccuugagaagaaaaugagcaauuacauacaguucaaguccaaaugccguauugagccuguauguuugcucnuacauggcagcccaggggccggaaaauccguggccaccaaccugauuggcagaucacucgcugaaaaacucaacagcucaguguacucccuaccaccagacccagaucacuuugauggcuacaaacagcaagcggucgugaucauggaugaucuaugccaaaauccugauggaaaagaugugucauuguucugucaaaugguuuccaguguggacuuuguaccaccgauggcugcgcuagaggagaaaggcauucuguucaccuccccguuuguccuggcaucaaccaaugcuggguccaucaaugcaccaacugugucagacagcagagcccucgcuaggagauuccacuuugacaugaacauugaagucauuuccauguacagucaaaauggcaagaucaacaugcccaugucaguuaagacgugugaugaagaguguuguccagucaacuucaagaggugcugcccgcugguguguggaaaggccaugcaguucauugacagaagaacucaaguuagauacucgcuggacaugcuaguuacugagauguuuagggaguacaaccacagacacagugugggagccacccuugaggcucuguuccaagggccaccagucuacagagagaucaaaauuagugucgcaccagagacaccaccaccaccagcuauugcugacuuacugaaaucaguggacagugaagcugugagagaguacugcaaagaaaagggauggcuugugccagagaucaacuccacccuacaaauugagaagcaugugagccgggcauucaucugucugcaagcacuaaccacguuuguuucaguugcuggaauaauauacauuauuuacaagcuauuugcagguuuccaaggcgcauacacagggaugcccaaccagaaacccaaggugcccacccugagacaagccaaagugcaaggcccagcguuugaguuugcuguggcgaugaugaagaggaacuccaguacagugaaaaccgaguacggugaguucaccaugcuuggcauuuaugacaggugggcgguguuaccacgccacgccaaaccuggcccaaccaucuugaugaaugaccaggaagucggcguguuggaugccaaggaacuaguggauaaggaugggacaaaccuagaacugacacuccugaagcucaacaguaaugagaaguucagagacaucagaggguuccuagccaaagaagagguugaggugaaugaagcuguccuagcaauaaacacaagcaaguuccccaacauguacauaccagugggccaggugacugacuacggguuccugaaccugggugggacgcccacuaagagaaugcucauguacaacuuccccacuagagcaggucaguguggugguguccucauguccacugggaaaguccuggggauacauguuggugggaauggucaucaaggguucucagcagcacuccucaagcacuacuucaacgaugaacaaggugaaauagaguucauugagagcucaaaggacgcgggguucccuaucaucaacacacccagcaagaccaaacuggaaccaagugucuuccaccaguguuugaaggcaacaaagaacccagcaguccucagaaauggugauccacgacucaaagccaacuuugaggaggccaucuucuccaaauacauuggcaaugucaacacgcauguggaugaguacauguuggaagcuguggaccauuaugcaggacaacuggcuacucuggacaucagcacggaaccaaugaagcuggaggaugccguguaugguacagaggggcuggaagcacuagaccuaacaaccagugcaggcuacccuuauguugcccugggcaucaagaagagagacauccuaucuaagaagaccagggaccucacuaaguugaaagaaugcauggacaaguauggccuaaaccugccaaugguaaccuaugugaaagaugagcucagaucugcagagaagguggccaaaggaaaauccaggcuuauugaagcuuccaguuugaaugacucaguggcaaugagacagacauuuggaaaccuguacaaaaccuuccaccucaacccaggcauugugacgggcagugcaguugggugugacccagaucuguuuuggagcaagauaccagucauguuggauggacaucucauagcuuuugauuacucaggcuaugaugcuagccucagcccagugugguuugcaugucugaaacugcuccuagagaagcuuggguacacacacaaggaaacaaacuacauagauuaccucugcaacucccaccaccuguacagagacaaacacuacuuugugcgaggugguaugccaucaggguguucuggcaccagcaucuuuaacucaaugauuaacaacaucauaaucaggacacucaugcugaaaguguacaagggcauugacuuggaccaauucaggauuauugccuauggugaugaugugauugcuuccuacccguggcccauugaugcuucccugcuagcugaagcaggaaaagauuaugguuugaucaugacaccagcagauaaaggagagugcuucaaugaagucaacuggacgaaugucaccuuccugaaaagguacuuuagagcagaugagcaauacccauuccugguccacccuguuaugcccaugaaagacauccaugaaucuauuagauggaccaaagauccaaagaacacccaagaucaugugcgcucgcugugccuauuggcuuggcacaauggggagcacgaauaugaggaguucauucgcaaaaucagaaagcgugccaguuggacgcuguuugacccuaccugcguuuucaacccugcgcaggaagugguuggacuccuuuuaaaauaaagcacaauuuaguaaauuugaauuggcuuaacccuaccgcacuaaccgaacuagauaacggugcgguagggguaaauucuccgcauucggugcggucgagg

SEQ ID NO: 3 - RNA, 7427 nt, Enterovirus sp. Echo 7
  CDS (743)-(7327): Modified virus after propagation for 12 months
uuaaaacagccuguggguuguucccacccacagggcccacugggcgcuagcacacugguaucacgguacccuugugcgccuguuuuaucuuccccuccccacuguaacuuagaagaaugacauaaacggucaacagauagcucaguacaccaacugagccccgaccaagcacuucuguuaccccggaccgaguaacaauaggcugcucgcgcggcugaaggugaaaacguucguuacccggccaauuacuucgagaaaccuaguaccaccaugaagguugcgcagcguuucgcuccgcacaaccccaguguagaucaggucgaugagucaccgcacuccccacgggcgaccguggcgguggcugcgcuggcggccugccuauggggcaacccaugggacgcuucaauacugacauggugcgaagagucuauugagcuaauugguaguccuccggccccugaaugcggcuaauccuaacugcggggcaagugcccacaaaccaguggguggcuugucguaacggguaacccugcagcggaaccgacuacuuuggguguccguguuuccuuuuauucuuauucuggcugcuuauggugacaauugagagauuguugccauauagcuauuggauuggccaucuggugaguaacagagcaaucauauuccucuuuguuggauuuauaccacuugauuccacuaguuacaacacucugcuacauauuauuugcuuaaauacaagaagaugggagcacaaguaucgacacaaaagacuggugcacacgagaccgguuugagcgcuaacggacacucuaucauucacuauaccaacaucaacuacuacaaagaugcagcauccaacucagccaacaggcaggauuucacccaggauccagguaaguucacugaaccggucaaggauaucaugaucaaaucgaugcccgcccuaaacucaccguccgcggaggagugcggguacagcgacagggugagaucccuaacgyucggcaacucaaccauuaccacucaagaaagugcaaacguaguuguuggcuauggcagguggccagaguacuugaaagaugaagaagcuacugcggaagaucagccaacacaacccgauguagccacaugcagguucuacacguuggaauccguccagugggagaaaaauagcgcuggauggugguggaaguuccccgaagcacuuaaggacaugggccucuuuggucagaacaugcuuuaccacuaucucgguagagcaggcuacacuauacaugugcagugcaacgcauccaaauuucaucagggcugucuacuuguugucuguguaccugaagcugagaugggguguucccagacggacaaagagguugcugcgaugaaccucacgaagggugaaacggcgcacaaguuugaaccaaccaaaaccacaggcggccacacagugcaauccauagugugcaacgcggguaugggcaucggcguggggaaccucaccaucuacccucaccaguggaucaacuugcgcacuaauaacugcgcuacaauugugaugccguauauaaauucaguacccauggauaacauguuuaggcacuacaauuucacgcuaauggugaucccauuugcaccccuggauuacaaugcccaagcaucugaguacguaccuguaacugucacaauagccccaaugugugcagaauacaaugguuuraggcuggcuuaccagcaagggcugccagugcuaaauacaccgggaagcaaucaguuuaugacaucggaugauuuucaauccccuucggcuaugccacaauuugaugugacuccgcacauggacaucccaggugaagugcacaaccucauggagauugcagaaguugauucggugguaccuguuaacaacacugcggccaaucugcaaagcauggacgcauaucacauagaggugaacgcaggaaaucaccaaggugaaaagauauucgcuuuccagauacaacccgggcuggauucaguguuuaagagaacacugcuaggugaagugcucaauuauuacgcgcacuggucagggagcauuaagcuaacauucacauuuugugguucagcaauggccacgggcaagcuacucuuagcauacuccccaccuggcgccgauguaccggcuagcagaaagcaggcaaugmugggaacccauaucaucugggacuuagggcugcaauccaguugcguucuauguauuccauggaucagucagacacauuaucgccuagugcaacaggaugaguacaccagcgccggcaaugucaccugcugguaucagacagguauagugguuccacccggcacacccaacaagugugucguccugugcuuugugucagcguguaaugacuucuccgugcgcaugcugcgugacacaccauucaucggccaaacaacacugcuacaaggugauacggacguggccgucaacaaugcaguagccaggguagcugauacaauugccagugggcccagcaacuccacuagcauuccugcacuaaccgcaguugagacugggcacacaucacagguagagccuagugauacaaugcaaacacggcauguaaagaacuaccauucgcgaucugaaucaacaauagagaacuuccuuagccggucggccuguguauauwuugaagasuacuuuaccaaagaucaagacagcgccaauagguacaugucauggacuauaaaugcuagaaggauggugcaauugaggcgaaaguuugaacuguucacauacaugcgguuugauauggagaucacauuuguuaucacuaguagacaacugccugggacuagcaucgcgcaagacaugccgccacugacacaccaaaucauguauauacccccuggugguccaruaccaaacagugugaccgauuuugcauggcaaacuucgacuaauccaaguaucuuuuggacugagggcaaugcccccccgcguauguccauaccauuuauaagcauagggaaugcauacagcaacuuuuaugacggauggucgcacuucucacaaaaugggguauacggcuacaaugcauuaaacaacaugggcaaauuauacgcacgccaugugaacaaagacacaccguaccagauguccaguacgauucguguguacuuuaaacccaaacauaucagagugugggugccaagaccaccacguuugugccccuauauuaaaucuaguaacguuaacuuugacccaaccaaccuaacugauucaagaucaaguauaacauaugugccagacacuauccguccggaaguccguacagcuggaaaauucggccaccaguccggugcuguuuacguggguaauuacagaauagugaacaggcaccucgccacgcacaacgacuggcaaaacugugugugggaagacuacaacagagaccuccuugugagcaccacuacagcccaugggugugacacuauagccagaugucagugcacagcaggcguauauuuuugugccucaaggaacaaacauuacccagucaccuucgaggggccaggcuugguggaaguucaggagagcgaguacuacccaaaaagauaucagucccacgugcuucuagcugcaggauuuucugaaccgggcgauuguggcggaauccucagaugucaacacggcgugaucgguaucgucaccauggguggagagggggucguuggguuugccgacgucagagaccuacugugguuagaggaugaugccauggaacagggcguaagagacuauguugaacaacuaggaaaugcuuucggcucagguuucaccaaucaaauuugugaacaggucaaccuccucaaagagucauugguuggacaggauucuauucuggaaaaaucccuuaaggcucuaguuaagauuaucucagcacuggucguuguagugagaaaucacgaugaucucauaacgguuaccgccacucuagcuuuaauugguugcaccucuucuccguggcgguggcucaagcagaaggugucacaauauuauggaauacccagggccgagcgacaaaacaauagcuggcucaagaaguuuacugagaugaccaacgccugcaagggcauggaguggauagccauaaaaauucaaaaguuuauugaguggcuuaaagucaagauucugccggaagugaaggaaaaacacgaguuccucaacaggcuaaagcaauuaccacuccuagagagccagauugcaaccauagagcagagugcaccaucgcagagugaucaagagcaacucuucuccaacguccaguacuucgcccauuauugcagaaaguaugcgccauuguacgcugccgaggcgaagagaguguucucacuugagaagaaaaugagcaacuacauacaguucaaguccaaaugccguauugagccuguaugcuuacuccuacauggcagcccaggggccggaaaguccguggccaccaacuugauuggcagaucccucgcagaaaaacucaacagcucuguauacucccuaccaccagaccccgaccacuuugacggcuacaagcagcaagcggucgugaucauggaugacuuaugccaaaauccugauggaaaagaugucucacuauuuugucagaugguuucuagcguggacuuuguaccaccgauggcugcgcuagaggaaaaaggaauccuauuuaccuccccguucguguuggcaucaaccaacgcuggguccaucaaugcacccacugugucugacagcagagcgcucgcuaggagauuccacuuugacaugaacauugaagucauuucuauguacagucaaaacggcaagaucaacaugcccaugucaguuaaaacaugugaugaagaguguuguccaguuaacuucaaaaggugcugcccguuggugugugggaaggcyaugcaauucauugauaggagaacucaaguuagauauucgcuggacaugcuaguuacugaaauguuuagggaguauaaccauagacacagugugggagccacucuugaagcucuguuccaagggccaccagucuacagagagaucaaaaucagcgucgccccagagacacccccaccaccagcuauugcugauuuacugaaaucaguggacagugaagcugugagggaauacugcaaggagagaggguggcuugugccagagaucaauucuacccuacaaauagagaagcaugugaguagagcauucauauguuuacaagcccuaaccacguuuguuucaguugcugguauaauauacauuauuuacaaauuauuugcagguuuccaaggcgccuacacagggaugcccaaccagaaaccuaaggugcccacccugagacaggccaaaguacagggcccagcguuugaguucgcuguggcgaugaugaaaaggaacgccaguacaguaaaaaccgaguacggugaauucaccaugcuuggcauuuacgacaagugggcgguguuaccgcgccacgccaagccuggccccaccaucuugaugaaugaucaggaagucggcguguuggaugccaaggaacuaguugauaaagaugggacaaaucuagaauugacucuccugaagcucaaccguaacgaaaaguucagagauauuaggggguuucuagcaagagaagagguugaagugaaugaagcuguccuagcaauaaauacaagcaaauucccuaacauguacauaccagugggccaggugacugacuacggguuucugaaccugggagggacucccacgaagagaaugcucauguauaacuucccaacuagagcaggucaguguggagguguccucaugucaacagggaaaguccugggaauacauguaggagggaauggacaucaaggguucucagcggcacuccucaggcacuacuucaacgaggagcagggugaaauagaauucauugagagcucaaaggacgcgggauucccugugaucaacacucccaguaagacaaaauuggaaccaaguguguuucaccagguguucgagggcaacaaggaaccagcgguccuuagaaauggggacccacgacucaaagccaacuucgaggaagcaaucuucuccaaguacauuggcaaugucaacacgcauguagaugaguacauguuggaggcuguggaccauuaugcaggacaacuagcuacucuggacaucaguacggagcccaugaagcuagaggacgccguguaugguacagaggggcuggaagcacuagaccuaaccaccagugcaggcuacccuuacguggcccugggcaucaagaaaagagauauucuaucuaagaagacuaaagaccucacuaaguugaaggaaugcauggacaaauauggccuaaauuugccaaugguaaccuacgucaaagaugaguugagaucugcugagaagguggccaagggaaaauccaggcuuauugaggcuucuagucucaaugacucaguagcaaugaggcaaacauuuggaaauuuauauaagaccuuucaccucaacccgggcaucguuacgggcagugcuguugggugugauccagauguguuuuggagcaagaucccuguuaugcuugauggacaucucauagcuuuugacuauucaggcuaugacgcuagccucagcccagugugguuugcauguuugaaacuucuccuagagaaacuaggguauacaaacaaggaaacaaacuacauagauuaccucuguaauucccaucaccuguauagagacaagcacuacuuuguaagaggcgguaugccaucaggguguucaggcaccagcauauuuaauuccaugauuaacaacaucauaaucaggacucucaugcugaagguuuauaaaggcauugauuuggaccaauucagaaugauugccuauggggaugaugugauugcuuccuauccguggccuaucgaugcuucgcuguuagcugaagcaggaaaagauuaugguuuaaucaugaccccagcagacaaaggcgagugcuucaacgagguaaccuggacgaaugugaccuuucugaaaagguacuuuagggcagaugagcaauacccauuucugguccauccuguuaugccaaugaaggacauacaugaguccauuagguggaccaaagaucccaagaacacacaggaucaugugcgcucgcugugccuauuggcuuggcacaacggggagcaagaauaugaggaguuuauucgcaagaucagaagcgugcccguugggcgcugcuugacccuacccgcuuuuucaacacugcgcaggaaguggcuggacuccuuuuaaaauuagagcauaauuaguaaaucauaauuggcuuaacccuaccgcaugaaccgaacuugauaaaagugcgguagggguaaauucuccgcauucggugcgg

SEQ ID NO: 4 - protein, 2194 aa, Enterovirus sp. Echo 7
  UNSURE 16, 404, 954, 1065: Amino acid sequence of the modified virus
MGAQVSTQKTGAHETXLSANGHSIIHYTNINYYKDAASNSANRQDFTQDPGKFTEPVKDIMIKSMPALNSPSAEECGYSDRVRSLTLGNSTITTQESANVVVGYGRWPEYLKDEEATAEDQPTQPDVATCRFYTLESVQWEKNSAGWWWKFPEALKDMGLFGQNMLYHYLGRAGYTIHVQCNASKFHQGCLLVVCVPEAEMGCSQTDKEVAAMNLTKGETAHKFEPTKTTGGHTVQSIVCNAGMGIGVGNLTIYPHQWINLRTNNCATIVMPYINSVPMDNMFRHYNFTLMVIPFAPLDYNAQASEYVPVTVTIAPMCAEYNGLRLAYQQGLPVLNTPGSNQFMTSDDFQSPSAMPQFDVTPHMDIPGEVHNLMEIAEVDSVVPVNNTAANLQSMDAYHIEVNXGNHQGEKIFAFQIQPGLDSVFKRTLLGEVLNYYAHWSGSIKLTFTFCGSAMATGKLLLAYSPPGADVPASRKQAMMGTHIIWDLGLQSSCVLCIPWISQTHYRLVQQDEYTSAGNVTCWYQTGIVVPPGTPNKCVVLCFVSACNDFSVRMLRDTPFIGQTTLLQGDTDVAVNNAVARVADTIASGPSNSTSIPALTAVETGHTSQVEPSDTMQTRHVKNYHSRSESTIENFLSRSACVYIEEYFTKDQDSANRYMSWTINARRMVQLRRKFELFTYMRFDMEITFVITSRQLPGTSIAQDMPPLTHQIMYIPPGGPVPNSVTDFAWQTSTNPSIFWTEGNAPPRMSIPFISIGNAYSNFYDGWSHFSQNGVYGYNALNNMGKLYARHVNKDTPYQMSSTIRVYFKPKHIRVWVPRPPRLCPYIKSSNVNFDPTNLTDSRSSITYVPDTIRPEVRTAGKFGHQSGAVYVGNYRIVNRHLATHNDWQNCVWEDYNRDLLVSTTTAHGCDTIARCQCTAGVYFCASRNKHYPVTFEGPGLVEVQESEYYPKRXQSHVLLAAGFSEPGDCGGILRCQHGVIGIVTMGGEGVVGFADVRDLLWLEDDAMEQGVRDYVEQLGNAFGSGFTNQICEQVNLLKESLVGQDSILEKSLKALVKIISALVXVVRNHDDLITVTATLALIGCTSSPWRWLKQKVSQYYGIPRAERQNNSWLKKFTEMTNACKGMEWIAIKIQKFIEWLKVKILPEVKEKHEFLNRLKQLPLLESQIATIEQSAPSQSDQEQLFSNVQYFAHYCRKYAPLYAAEAKRVFSLEKKMSNYIQFKSKCRIEPVCLLLHGSPGAGKSVATNLIGRSLAEKLNSSVYSLPPDPDHFDGYKQQAVVIMDDLCQNPDGKDVSLFCQMVSSVDFVPPMAALEEKGILFTSPFVLASTNAGSINAPTVSDSRALARRFHFDMNIEVISMYSQNGKINMPMSVKTCDEECCPVNFKRCCPLVCGKAMQFIDRRTQVRYSLDMLVTEMFREYNHRHSVGATLEALFQGPPVYREIKISVAPETPPPPAIADLLKSVDSEAVREYCKERGWLVPEINSTLQIEKHVSRAFICLQALTTFVSVAGIIYIIYKLFAGFQGAYTGMPNQKPKVPTLRQAKVQGPAFEFAVAMMKRNASTVKTEYGEFTMLGIYDKWAVLPRHAKPGPTILMNDQEVGVLDAKELVDKDGTNLELTLLKLNRNEKFRDIRGFLAREEVEVNEAVLAINTSKFPNMYIPVGQVTDYGFLNLGGTPTKRMLMYNFPTRAGQCGGVLMSTGKVLGIHVGGNGHQGFSAALLRHYFNEEQGEIEFIESSKDAGFPVINTPSKTKLEPSVFHQVFEGNKEPAVLRNGDPRLKANFEEAIFSKYIGNVNTHVDEYMLEAVDHYAGQLATLDISTEPMKLEDAVYGTEGLEALDLTTSAGYPYVALGIKKRDILSKKTKDLTKLKECMDKYGLNLPMVTYVKDELRSAEKVAKGKSRLIEASSLNDSVAMRQTFGNLYKTFHLNPGIVTGSAVGCDPDVFWSKIPVMLDGHLIAFDYSGYDASLSPVWFACLKLLLEKLGYTNKETNYIDYLCNSHHLYRDKHYFVRGGMPSGCSGTSIFNSMINNIIIRTLMLKVYKGIDLDQFRMIAYGDDVIASYPWPIDASLLAEAGKDYGLIMTPADKGECFNEVTWTNVTFLKRYFRADEQYPFLVHPVMPMKDIHESIRWTKDPKNTQDHVRSLCLLAWHNGEQEYEEFIRKIRSVPVGRCLTLPAFSTLRRKWLDSF

SEQ ID NO: 5 - protein, 2196 aa, Enterovirus sp. Echo 7
  UNSURE 16, 404, 1236: amino acid sequence of the unmodified virus
MGAQVSTQKTGAHETXLSANGSSIIHYTNINYYKDAASNSANRQDFTQDPGKFTEPVKDIMIKSMPALNSPTVEECGYSDRVRSITLGNSTITTQESANVVVGYGGWPEYLKDEEATAEDQPTQPDVATCRFYTLESVQWEKNSAGWWWKFPEALKDMGLFGQNMHYHYLGRAGYTIHVQCNASKFHQGCLLVVCVPEAEMGCSKVDGTVNEQELTEGETDMKLEPTRTTGVRRVQSAVYNAGMGVGVGNLTIFPHQWINLRTNNCATIVMPYINSVPMDNMFRHYNFTLMMIPFAPLDYTNQASTYVPITVTIAPMCAEYNGLRLVTSQGLPVMNTPGSNQFLTSDDFQSPSAMPQFDVTPDMDIPGEVNNLMEIAEVDSVVPVNNNEANLKSMDAYRIPVNXGNQQGEKIFGFQIQPGLDSVFKRTLLGEMLNYYTHWSGSIKLTFMFCGSAMATGKLLLAYSPPGADVPTSRKEAMLGTHVIWDFGLQSSCVLCVPWISQTHYRLVQQDEYTGAGYITCWYQTSIVVPPGTPKKCVILCFVSACNDFSVSMLSDTPFIGQTALLQSPVEEAEENAVARVADTIASGPSNSESVPALTAVETGHTSQVVPSDTMQTRHVKNYHSRSESTIENFLSRSACVYIEEYYTNTETRQNLYMLPTINTRWMVQLRRKFEMFTYMRFDMEITFVITSRQLHRTSMPQDMPVLTHQIMYVPPGGPVPNSVDDYAWQTSTNPSVFWTEGNAPPRMSIPFISIGNAYSNFYDGSSHFLQYGVYGYNTLNNMGKLYVRHVNNHTPYQMTSTVSVYFKPKHVRAWVPRPPRLCPYKNAWNVNFEPTNVTDSRSSITYIPETVKPDLSKAGAFGHQSGAVYVGNYRVVNRHLATHNDWQNCVWEDYNRDLLVSTTTAHGCDTIARCQCTTGVYFCASRNKHYPVTFEGPGLVEVQESEYYPKRYQSHVLLAAGFSEPGDCGGILRCEHGVIGIVTMGGEGVVGFADVRDLLWLEDDAMEQGVRDYVEQLGNAFGSGFTNQICEQVNLLKESLVGQDSILEKSLKALVKIISALVIVVRNHDDLITVTATLALIGCTSSPWRWLKQKVSQYYGIPMAERQNNGWLKKFTEMTNACKGMEWIAIKIQKFIEWLKVKIYQKCRKNMSSSTDYNNYHSWKSQIATIEQSAPSQSDQEQLFSNVQYFAHYCRKYAPLYAAEAKRVFSLEKKMSNYIQFKSKCRIEPVCLLXHGSPGAGKSVATNLIGRSLAEKLNSSVYSLPPDPDHFDGYKQQAVVIMDDLCQNPDGKDVSLFCQMVSSVDFVPPMAALEEKGILFTSPFVLASTNAGSINAPTVSDSRALARRFHFDMNIEVISMYSQNGKINMPMSVKTCDEECCPVNFKRCCPLVCGKAMQFIDRRTQVRYSLDMLVTEMFREYNHRHSVGATLEALFQGPPVYREIKISVAPETPPPPAIADLLKSVDSEAVREYCKEKGWLVPEINSTLQIEKHVSRAFICLQALTTFVSVAGIIYIIYKLFAGFQGAYTGMPNQKPKVPTLRQAKVQGPAFEFAVAMMKRNSSTVKTEYGEFTMLGIYDRWAVLPRHAKPGPTILMNDQEVGVLDAKELVDKDGTNLELTLLKLNSNEKFRDIRGFLAKEEVEVNEAVLAINTSKFPNMYIPVGQVTDYGFLNLGGTPTKRMLMYNFPTRAGQCGGVLMSTGKVLGIHVGGNGHQGFSAALLKHYFNDEQGEIEFIESSKDAGFPIINTPSKTKLEPSVFHQCLKATKNPAVLRNGDPRLKANFEEAIFSKYIGNVNTHVDEYMLEAVDHYAGQLATLDISTEPMKLEDAVYGTEGLEALDLTTSAGYPYVALGIKKRDILSKKTRDLTKLKECMDKYGLNLPMVTYVKDELRSAEKVAKGKSRLIEASSLNDSVAMRQTFGNLYKTFHLNPGIVTGSAVGCDPDLFWSKIPVMLDGHLIAFDYSGYDASLSPVWFACLKLLLEKLGYTHKETNYIDYLCNSHHLYRDKHYFVRGGMPSGCSGTSIFNSMINNIIIRTLMLKVYKGIDLDQFRIIAYGDDVIASYPWPIDASLLAEAGKDYGLIMTPADKGECFNEVNWTNVTFLKRYFRADEQYPFLVHPVMPMKDIHESIRWTKDPKNTQDHVRSLCLLAWHNGEHEYEEFIRKIRKRASWTLFDPTCVFNPAQEVVGLLLK

SEQ ID NO: 6 - DNA, 20 bp, Artificial sequence
  Primer Eo7-1F
ttaaaacagcctgtgggttg

SEQ ID NO: 7 - DNA, 22 bp, Artificial sequence
  Primer Eo7-1R
gaaacacggacacccaaagtag

SEQ ID NO: 8 - DNA, 20 bp, Artificial sequence
  Primer Eo7-2F
ccatgggacgcttcaatact

SEQ ID NO: 9 - DNA, 20 bp, Artificial sequence
  Primer Eo7-2R
gcaccagtcttttgtgtcga

SEQ ID NO: 10 - DNA, 25 bp, Artificial sequence
  Primer Eo7-3F
cgactactttgggtgtccgtgtttc

SEQ ID NO: 11 - DNA, 23 bp, Artificial sequence
  Primer Eo7-3R
tcdggraayttccaccaccaccc

SEQ ID NO: 12 - DNA, 20 bp, Artificial sequence
  Primer Eo7-4F
cgacagggtgagatccctaa

SEQ ID NO: 13 - DNA, 20 bp, Artificial sequence
  Primer Eo7-4R
tttcacccttcgtgaggttc

SEQ ID NO: 14 - DNA, 20 bp, Artificial sequence
  Primer Eo7-5F
gcatcyaarttycaycargg

SEQ ID NO: 15 - DNA, 20 bp, Artificial sequence
  Primer Eo7-5R
cacatkggkgcaatsgtgac

SEQ ID NO: 16 - DNA, 20 bp, Artificial sequence
  Primer Eo7-6F
gtggatcaacttgcgcacta

SEQ ID NO: 17 - DNA, 20 bp, Artificial sequence
  Primer Eo7-6R
aaattgtggcatagccgaag

SEQ ID NO: 18 - DNA, 20 bp, Artificial sequence
  Primer Eo7-7F
gtcacsattgcmccmatgtg

SEQ ID NO: 19 - DNA, 23 bp, Artificial sequence
  unsure 4: Primer Eo7-7R
cttnatrctycctgaccagtgtg

SEQ ID NO: 20 - DNA, 20 bp, Artificial sequence
  Primer Eo7-8F
aagcatggacgcatatcaca

SEQ ID NO: 21 - DNA, 20 bp, Artificial sequence
  Primer Eo7-8R
gatatgggttcccacattgc

SEQ ID NO: 22 - DNA, 23 bp, Artificial sequence
  unsure 20: Primer Eo7-9F
cacactggtcaggragyatnaag

SEQ ID NO: 23 - DNA, 20 bp, Artificial sequence
  Primer Eo7-10F
caagtgtgtcgtcctgtgct

SEQ ID NO: 24 - DNA, 20 bp, Artificial sequence
  Primer Eo7-9R
cctattggcgctgtcttgat

SEQ ID NO: 25 - DNA, 20 bp, Artificial sequence
  Primer Eo7-11F
accaaagatcaagacagcgc

SEQ ID NO: 26 - DNA, 20 bp, Artificial sequence
  Primer Eo7-11R
ttggcacccacactctgata

SEQ ID NO: 27 - DNA, 20 bp, Artificial sequence
  Primer Eo7-12F
accagtccggtgctgtttac

SEQ ID NO: 28 - DNA, 23 bp, Artificial sequence
  Primer Eo7-12R
tcccayacacarttytgccagtc

SEQ ID NO: 29 - DNA, 23 bp, Artificial sequence
  Primer Eo7-13F
caraaytgtgtgtgggaagacta

SEQ ID NO: 30 - DNA, 27 bp, Artificial sequence
  Primer Eo7-13R
ccctgytccatkgcttcatcytcyarc

SEQ ID NO: 31 - DNA, 20 bp, Artificial sequence
  Primer Eo7-14F
ttacccagtcaccttcgagg

SEQ ID NO: 32 - DNA, 20 bp, Artificial sequence
  Primer Eo7-14R
tgtttttccttcacttccgg

SEQ ID NO: 33 - DNA, 27 bp, Artificial sequence
  unsure 16: Primer Eo7-15F
gttrgargatgatgcnatggarcargg

SEQ ID NO: 34 - DNA, 23 bp, Artificial sequence
  Primer Eo7-15R
tcaatacggyrtttgswcttgaa

SEQ ID NO: 35 - DNA, 20 bp, Artificial sequence
  Primer Eo7-16F
cctytrtaygcvgcygargc

SEQ ID NO: 36 - DNA, 23 bp, Artificial sequence
  Primer Eo7-17F
ttcaagwscaaayrccgtattga

SEQ ID NO: 37 - DNA, 23 bp, Artificial sequence
  Primer Eo7-16R
aaytgaatggcctthccacacac

SEQ ID NO: 38 - DNA, 23 bp, Artificial sequence
  unsure 21: Primer Eo7-18F
ctdgtgtgtggraaggcyatnca

SEQ ID NO: 39 - DNA, 23 bp, Artificial sequence
  Primer Eo7-18R
tatgctccytgraarcctgcaaa

SEQ ID NO: 40 - DNA, 20 bp, Artificial sequence
  Primer Eo7-19F
caagccctaaccacgtttgt

SEQ ID NO: 41 - DNA, 20 bp, Artificial sequence
  Primer Eo7-19R
acccgtagtcagtcacctgg

SEQ ID NO: 42 - DNA, 23 bp, Artificial sequence
  Primer Eo7-20F
tttgcaggmttycarggwgcata

SEQ ID NO: 43 - DNA, 23 bp, Artificial sequence
  Primer Eo7-20R
gcyctwgtgggraagttrtacat

SEQ ID NO: 44 - DNA, 20 bp, Artificial sequence
  Primer Eo7-21F
gtgttggatgccaaggaact

SEQ ID NO: 45 - DNA, 20 bp, Artificial sequence
  Primer Eo7-21R
atgggctccgatctgatgtc

SEQ ID NO: 46 - DNA, 26 bp, Artificial sequence
  Primer Eo7-22F
ttccccacwagrgcaggccartgygg

SEQ ID NO: 47 - DNA, 23 bp, Artificial sequence
  Primer Eo7-22R
ctccaaaabasrtcygggtcrca

SEQ ID NO: 48 - DNA, 20 bp, Artificial sequence
  Primer Eo7-23F
tgaaggaatgcatggacaaa

SEQ ID NO: 49 - DNA, 20 bp, Artificial sequence
  Primer Eo7-23R
atgggtattgctcatctgcc

SEQ ID NO: 50 - DNA, 23 bp, Artificial sequence
  Primer Eo7-24F
tgygacccrgaystvttttggag

SEQ ID NO: 51 - DNA, 22 bp, Artificial sequence
  Primer Eo7-24R
tcrtgdatdtcyttcatgggca

SEQ ID NO: 52 - DNA, 20 bp, Artificial sequence
  Primer Eo7-25F
cctggacgaatgtgaccttt

SEQ ID NO: 53 - DNA, 20 bp, Artificial sequence
  Primer Eo7-25R
ccctaccgcacttttatcca

SEQ ID NO: 54 - DNA, 23 bp, Artificial sequence
  Primer Eo7-26F
atccaygartchatyagrtggac

SEQ ID NO: 55 - DNA, 24 bp, Artificial sequence
  Primer Eo7-26R
ccgcaccgaatgcggagaatttac